European Patent Application EP 4 556 559 A1, published May 21, 2025. Title: Mutant microorganism of Corynebacterium genus producing L-glutamic acid and method for producing L-glutamic acid using the same. Applicant: DAESANG CORPORATION. The sequence listing filed with the application follows.

SEQUENCE LISTING (9 sequences)

SEQ ID NO: 1 - DNA, 1179 bp, synthetic construct
  source 1..1179: mol_type = other DNA
atgaccatcgacctgcagcgttccacccaaaacctcacccatgaggaaatcttcgaggcacacgagggcggaaagctctccattagttccactcgtccgctccgcgacatgcgcgatctttcccttgcttacaccccaggtgttgctcaggtttgtgaagcaatcaaagaagatccagaggttgcacgcacccacacgggcattggaaacaccgtcgcggttatttccgacggcaccgctgttcttggccttggcgatatcggacctcaggcatcccttcccgtcatggagggcaaggctcagctgttcagctctttcgctggtttgaaggctatccctatcgttttggatgttcacgatgttgacgctttggttgagaccatcgcagccatcgcgccttctttcggtgctatcaacttggaggacatctccgctcctcgttgcttcgaggtggagcgccgcctcatcgagcgtctcgatattccagttatgcacgatgaccagcacggcaccgctgtggttatcctcgctgcgctgcgcaactccctgaagctgctggatcgcaagatcgaagacctcaagattgttatttccggcgcaggcgcagcgggcgttgcagctgtagatatgttgaccaatgctggcgcaaccgacatcgtggttcttgattcccgaggcatcatccacgacagccgtgaggatctttccccagttaaggctgctctcgcggagaagaccaaccctcgtggcatcagcggtggcatcaatgaggctttcaccggcgcggacctgttcatcggcgtgtccggcggcaacatcggcgaggacgctctcaaactcatggcaccacagccaatcctgttcaccctggcgaacccaaccccagagatcgatcctgaactgtctcagaagtacggcgccatcgtcgcgaccggccgctctgacctgcctaaccagatcaacaacgtgctagcgttcccaggcattttcgccggcgctctcgcagccaaggccaagaagatcacccccgagatgaagctcgctgcagcagaggcaatcgccgacatcgcagctgaggacctcgaggtcggccgcatcgtaccgaccgccttgaatccccgcgtcgccccagcagtaaaggcagctgtccaggccgtcgccgaagcgcaaaacgcttag

SEQ ID NO: 2 - protein, 392 aa, synthetic construct
MTIDLQRSTQNLTHEEIFEAHEGGKLSISSTRPLRDMRDLSLAYTPGVAQVCEAIKEDPEVARTHTGIGNTVAVISDGTAVLGLGDIGPQASLPVMEGKAQLFSSFAGLKAIPIVLDVHDVDALVETIAAIAPSFGAINLEDISAPRCFEVERRLIERLDIPVMHDDQHGTAVVILAALRNSLKLLDRKIEDLKIVISGAGAAGVAAVDMLTNAGATDIVVLDSRGIIHDSREDLSPVKAALAEKTNPRGISGGINEAFTGADLFIGVSGGNIGEDALKLMAPQPILFTLANPTPEIDPELSQKYGAIVATGRSDLPNQINNVLAFPGIFAGALAAKAKKITPEMKLAAAEAIADIAAEDLEVGRIVPTALNPRVAPAVKAAVQAVAEAQNA

SEQ ID NO: 3 - DNA, 1179 bp, Corynebacterium sp.
  source 1..1179: mol_type = genomic DNA
atgaccatcgacctgcagcgttccacccaaaacctcacccatgaggaaatcttcgaggcacacgagggcggaaagctctccattagttccactcgtccgctccgcgacatgcgcgatctttcccttgcttacaccccaggtgttgctcaggtttgtgaagcaatcaaagaagatccagaggttgcacgcacccacacgggcattggaaacaccgtcgcggttatttccgacggcaccgctgttcttggccttggcgatatcggacctcaggcatcccttcccgtcatggagggcaaggctcagctgttcagctctttcgctggtttgaaggctatccctatcgttttggatgttcacgatgttgacgctttggttgagaccatcgcagccatcgcgccttctttcggtgctatcaacttggaggacatctccgctcctcgttgcttcgaggtggagcgccgcctcatcgagcgtctcgatattccagttatgcacgatgaccagcacggcaccgctgtggttatcctcgctgcgctgcgcaactccctgaagctgctggatcgcaagatcgaagacctcaagattgttatttccggcgcaggcgcagcgggcgttgcagctgtagatatgttgaccaatgctggcgcaaccgacatcgtggttcttgattcccgaggcatcatccacgacagccgtgaggatctttccccagttaaggctgctctcgcggagaagaccaaccctcgtggcatcagcggtggcatcaatgaggctttcaccggcgcggacctgttcatcggcgtgtccggcggcaacatcggcgaggacgctctcaaactcatggcaccacagccaatcctgttcaccctggcgaacccaaccccagagatcgatcctgaactgtctcagaagtacggcgccatcgtcgcgaccggccgctctgacctgcctaaccagatcaacaacgtgctagcgttcccaggcattttcgccggcgctctcgcagccaaggccaagaagatcacccccgagatgaagctcgctgcagcagaggcaatcgccgacatcgcagctgaggacctcgaggtcggccgcatcgtaccgaccgccttggatccccgcgtcgccccagcagtaaaggcagctgtccaggccgtcgccgaagcgcaaaacgcttag

SEQ ID NO: 4 - protein, 392 aa, Corynebacterium sp.
MTIDLQRSTQNLTHEEIFEAHEGGKLSISSTRPLRDMRDLSLAYTPGVAQVCEAIKEDPEVARTHTGIGNTVAVISDGTAVLGLGDIGPQASLPVMEGKAQLFSSFAGLKAIPIVLDVHDVDALVETIAAIAPSFGAINLEDISAPRCFEVERRLIERLDIPVMHDDQHGTAVVILAALRNSLKLLDRKIEDLKIVISGAGAAGVAAVDMLTNAGATDIVVLDSRGIIHDSREDLSPVKAALAEKTNPRGISGGINEAFTGADLFIGVSGGNIGEDALKLMAPQPILFTLANPTPEIDPELSQKYGAIVATGRSDLPNQINNVLAFPGIFAGALAAKAKKITPEMKLAAAEAIADIAAEDLEVGRIVPTALDPRVAPAVKAAVQAVAEAQNA

SEQ ID NO: 5 - DNA, 5719 bp, synthetic construct
  source 1..5719: mol_type = other DNA
tgccgcaagcactcagggcgcaagggctgctaaaggaagcggaacacgtagaaagccagtccgcagaaacggtgctgaccccggatgaatgtcagctactgggctatctggacaagggaaaacgcaagcgcaaagagaaagcaggtagcttgcagtgggcttacatggcgatagctagactgggcggttttatggacagcaagcgaaccggaattgccagctggggcgccctctggtaaggttgggaagccctgcaaagtaaactggatggctttcttgccgccaaggatctgatggcgcaggggatcaagatctgatcaagagacaggatgaggatcgtttcgcatgattgaacaagatggattgcacgcaggttctccggccgcttgggtggagaggctattcggctatgactgggcacaacagacaatcggctgctctgatgccgccgtgttccggctgtcagcgcaggggcgcccggttctttttgtcaagaccgacctgtccggtgccctgaatgaactccaagacgaggcagcgcggctatcgtggctggccacgacgggcgttccttgcgcagctgtgctcgacgttgtcactgaagcgggaagggactggctgctattgggcgaagtgccggggcaggatctcctgtcatctcaccttgctcctgccgagaaagtatccatcatggctgatgcaatgcggcggctgcatacgcttgatccggctacctgcccattcgaccaccaagcgaaacatcgcatcgagcgagcacgtactcggatggaagccggtcttgtcgatcaggatgatctggacgaagagcatcaggggctcgcgccagccgaactgttcgccaggctcaaggcgcggatgcccgacggcgaggatctcgtcgtgacccatggcgatgcctgcttgccgaatatcatggtggaaaatggccgcttttctggattcatcgactgtggccggctgggtgtggcggaccgctatcaggacatagcgttggctacccgtgatattgctgaagagcttggcggcgaatgggctgaccgcttcctcgtgctttacggtatcgccgctcccgattcgcagcgcatcgccttctatcgccttcttgacgagttcttctgagcgggactctggggttcgctagaggatcgatcctttttaacccatcacatatacctgccgttcactattatttagtgaaatgagatattatgatattttctgaattgtgattaaaaaggcaactttatgcccatgcaacagaaactataaaaaatacagagaatgaaaagaaacagatagattttttagttctttaggcccgtagtctgcaaatccttttatgattttctatcaaacaaaagaggaaaatagaccagttgcaatccaaacgagagtctaatagaatgaggtcgaaaagtaaatcgcgcgggtttgttactgataaagcaggcaagacctaaaatgtgtaaagggcaaagtgtatactttggcgtcaccccttacatattttaggtctttttttattgtgcgtaactaacttgccatcttcaaacaggagggctggaagaagcagaccgctaacacagtacataaaaaaggagacatgaacgatgaacatcaaaaagtttgcaaaacaagcaacagtattaacctttactaccgcactgctggcaggaggcgcaactcaagcgtttgcgaaagaaacgaaccaaaagccatataaggaaacatacggcatttcccatattacacgccatgatatgctgcaaatccctgaacagcaaaaaaatgaaaaatatcaagtttctgaatttgattcgtccacaattaaaaatatctcttctgcaaaaggcctggacgtttgggacagctggccattacaaaacgctgacggcactgtcgcaaactatcacggctaccacatcgtctttgcattagccggagatcctaaaaatgcggatgacacatcgatttacatgttctatcaaaaagtcggcgaaacttctattgacagctggaaaaacgctggccgcgtctttaaagacagcgacaaattcgatgcaaatgattctatcctaaaagaccaaacacaagaatggtcaggttcagccacatttacatctgacggaaaaatccgtttattctacactgatttctccggtaaacattacggcaaacaaacactgacaactgcacaagttaacgtatcagcatcagacagctctttgaacatcaacggtgtagaggattataaatcaatctttgacggtgacggaaaaacgtatcaaaatgtacagcagttcatcgatgaaggcaactacagctcaggcgacaaccatacgctgagagatcctcactacgtagaagataaaggccacaaatacttagtatttgaagcaaacactggaactgaagatggctaccaaggcgaagaatctttatttaacaaagcatactatggcaaaagcacatcattcttccgtcaagaaagtcaaaaacttctgcaaagcgataaaaaacgcacggctgagttagcaaacggcgctctcggtatgattgagctaaacgatgattacacactgaaaaaagtgatgaaaccgctgattgcatctaacacagtaacagatgaaattgaacgcgcgaacgtctttaaaatgaacggcaaatggtacctgttcactgactcccgcggatcaaaaatgacgattgacggcattacgtctaacgatatttacatgcttggttatgtttctaattctttaactggcccatacaagccgctgaacaaaactggccttgtgttaaaaatggatcttgatcctaacgatgtaacctttacttactcacacttcgctgtacctcaagcgaaaggaaacaatgtcgtgattacaagctatatgacaaacagaggattctacgcagacaaacaatcaacgtttgcgccgagcttcctgctgaacatcaaaggcaagaaaacatctgttgtcaaagacagcatccttgaacaaggacaattaacagttaacaaataaaaacgcaaaagaaaatgccgatgggtaccgagcgaaatgaccgaccaagcgacgcccaacctgccatcacgagatttcgattccaccgccgccttctatgaaaggttgggcttcggaatcgttttccgggacgccctcgcggacgtgctcatagtccacgacgcccgtgattttgtagccctggccgacggccagcaggtaggccgacaggctcatgccggccgccgccgccttttcctcaatcgctcttcgttcgtctggaaggcagtacaccttgataggtgggctgcccttcctggttggcttggtttcatcagccatccgcttgccctcatctgttacgccggcggtagccggccagcctcgcagagcaggattcccgttgagcaccgccaggtgcgaataagggacagtgaagaaggaacacccgctcgcgggtgggcctacttcacctatcctgcccggctgacgccgttggatacaccaaggaaagtctacacgaaccctttggcaaaatcctgtatatcgtgcgaaaaaggatggatataccgaaaaaatcgctataatgaccccgaagcagggttatgcagcggaaaagcgctgcttccctgctgttttgtggaatatctaccgactggaaacaggcaaatgcaggaaattactgaactgaggggacaggcgagagacgatgccaaagagctcctgaaaatctcgataactcaaaaaatacgcccggtagtgatcttatttcattatggtgaaagttggaacctcttacgtgccgatcaacgtctcattttcgccaaaagttggcccagggcttcccggtatcaacagggacaccaggatttatttattctgcgaagtgatcttccgtcacaggtatttattcggcgcaaagtgcgtcgggtgatgctgccaacttactgatttagtgtatgatggtgtttttgaggtgctccagtggcttctgtttctatcagctcctgaaaatctcgataactcaaaaaatacgcccggtagtgatcttatttcattatggtgaaagttggaacctcttacgtgccgatcaacgtctcattttcgccaaaagttggcccagggcttcccggtatcaacagggacaccaggatttatttattctgcgaagtgatcttccgtcacaggtatttattcggcgcaaagtgcgtcgggtgatgctgccaacttactgatttagtgtatgatggtgtttttgaggtgctccagtggcttctgtttctatcagggctggatgatcctccagcgcggggatctcatgctggagttcttcgcccaccccaaaaggatctaggtgaagatcctttttgataatctcatgaccaaaatcccttaacgtgagttttcgttccactgagcgtcagaccccgtagaaaagatcaaaggatcttcttgagatcctttttttctgcgcgtaatctgctgcttgcaaacaaaaaaaccaccgctaccagcggtggtttgtttgccggatcaagagctaccaactctttttccgaaggtaactggcttcagcagagcgcagataccaaatactgttcttctagtgtagccgtagttaggccaccacttcaagaactctgtagcaccgcctacatacctcgctctgctaatcctgttaccagtggctgctgccagtggcgataagtcgtgtcttaccgggttggactcaagacgatagttaccggataaggcgcagcggtcgggctgaacggggggttcgtgcacacagcccagcttggagcgaacgacctacaccgaactgagatacctacagcgtgagctatgagaaagcgccacgcttcccgaagggagaaaggcggacaggtatccggtaagcggcagggtcggaacaggagagcgcacgagggagcttccagggggaaacgcctggtatctttatagtcctgtcgggtttcgccacctctgacttgagcgtcgatttttgtgatgctcgtcaggggggcggagcctatggaaaaacgccagcaacgcggcctttttacggttcctggccttttgctggccttttgctcacatgttctttcctgcgttatcccctgattctgtggataaccgtattaccgcctttgagtgagctgataccgctcgccgcagccgaacgaccgagcgcagcgagtcagtgagcgaggaagcggaagagcgcccaatacgcaaaccgcctctccccgcgcgttggccgattcattaatgcagctggcacgacaggtttcccgactggaaagcgggcagtgagcgcaacgcaattaatgtgagttagctcactcattaggcaccccaggctttacactttatgcttccggctcgtatgttgtgtggaattgtgagcggataacaatttcacacaggaaacagctatgacatgattacgccaagcttgcatgcctgcaggtcgactctagaggatccccgggtaccgagctcgaattcactggccgtcgttttacaacgtcgtgactgggaaaaccctggcgttacccaacttaatcgccttgcagcacatccccctttcgccagctggcgtaatagcgaagaggcccgcaccgatcgcccttcccaacagttgcgcagcctgaatggcgaatggcgataagctagcttcacgc

SEQ ID NO: 6 - DNA, 23 bp, synthetic construct
  source 1..23: mol_type = other DNA
catcgagcgtctcgatattccag

SEQ ID NO: 7 - DNA, 20 bp, synthetic construct
  source 1..20: mol_type = other DNA
cgcggggattcaaggcggtc

SEQ ID NO: 8 - DNA, 19 bp, synthetic construct
  source 1..19: mol_type = other DNA
gaccgccttgaatccccgc

SEQ ID NO: 9 - DNA, 23 bp, synthetic construct
  source 1..23: mol_type = other DNA
aacttctatgacctgcgtagcat